European Patent Application EP 4 650 369 A1, published November 19, 2025. Title: A fibrosis therapeutics comprises ICAM-1 inhibitor. Applicant: FNCT Biotech Inc. Application KR. The sequence listing filed with the application follows.

SEQUENCE LISTING (7 sequences)

SEQ ID NO: 1 - protein, 532 aa, Homo sapiens
MAPSSPRPALPALLVLLGALFPGPGNAQTSVSPSKVILPRGGSVLVTCSTSCDQPKLLGIETPLPKKELLLPGNNRKVYELSNVQEDSQPMCYSNCPDGQSTAKTFLTVYWTPERVELAPLPSWQPVGKNLTLRCQVEGGAPRANLTVVLLRGEKELKREPAVGEPAEVTTTVLVRRDHHGANFSCRTELDLRPQGLELFENTSAPYQLQTFVLPATPPQLVSPRVLEVDTQGTVVCSLDGLFPVSEAQVHLALGDQRLNPTVTYGNDSFSAKASVSVTAEDEGTQRLTCAVILGNQSQETLQTVTIYSFPAPNVILTKPEVSEGTEVTVKCEAHPRAKVTLNGVPAQPLGPRAQLLLKATPEDNGRSFSCSATLEVAGQLIHKNQTRELRVLYGPRLDERDCPGNWTWPENSQQTPMCQAWGNPLPELKCLKDGTFPLPIGESVTVTRDLEGTYLCRARSTQGEVTRKVTVNVLSPRYEIVIITVVAAAVIMGTAGLSTYLYNRQRKIKKYRLQQAQKGTPMKPNTQATPP

SEQ ID NO: 2 - protein, 453 aa, Homo sapiens
QTSVSPSKVILPRGGSVLVTCSTSCDQPKLLGIETPLPKKELLLPGNNRKVYELSNVQEDSQPMCYSNCPDGQSTAKTFLTVYWTPERVELAPLPSWQPVGKNLTLRCQVEGGAPRANLTVVLLRGEKELKREPAVGEPAEVTTTVLVRRDHHGANFSCRTELDLRPQGLELFENTSAPYQLQTFVLPATPPQLVSPRVLEVDTQGTVVCSLDGLFPVSEAQVHLALGDQRLNPTVTYGNDSFSAKASVSVTAEDEGTQRLTCAVILGNQSQETLQTVTIYSFPAPNVILTKPEVSEGTEVTVKCEAHPRAKVTLNGVPAQPLGPRAQLLLKATPEDNGRSFSCSATLEVAGQLIHKNQTRELRVLYGPRLDERDCPGNWTWPENSQQTPMCQAWGNPLPELKCLKDGTFPLPIGESVTVTRDLEGTYLCRARSTQGEVTRKVTVNVLSPRYE

SEQ ID NO: 3 - RNA, 1599 nt, Homo sapiens
  source 1..1599: mol_type = mRNA
atggctcccagcagcccccggcccgcgctgcccgcactcctggtcctgctcggggctctgttcccaggacctggcaatgcccagacatctgtgtccccctcaaaagtcatcctgccccggggaggctccgtgctggtgacatgcagcacctcctgtgaccagcccaagttgttgggcatagagaccccgttgcctaaaaaggagttgctcctgcctgggaacaaccggaaggtgtatgaactgagcaatgtgcaagaagatagccaaccaatgtgctattcaaactgccctgatgggcagtcaacagctaaaaccttcctcaccgtgtactggactccagaacgggtggaactggcacccctcccctcttggcagccagtgggcaagaaccttaccctacgctgccaggtggagggtggggcaccccgggccaacctcaccgtggtgctgctccgtggggagaaggagctgaaacgggagccagctgtgggggagcccgctgaggtcacgaccacggtgctggtgaggagagatcaccatggagccaatttctcgtgccgcactgaactggacctgcggccccaagggctggagctgtttgagaacacctcggccccctaccagctccagacctttgtcctgccagcgactcccccacaacttgtcagcccccgggtcctagaggtggacacgcaggggaccgtggtctgttccctggacgggctgttcccagtctcggaggcccaggtccacctggcactgggggaccagaggttgaaccccacagtcacctatggcaacgactccttctcggccaaggcctcagtcagtgtgaccgcagaggacgagggcacccagcggctgacgtgtgcagtaatactggggaaccagagccaggagacactgcagacagtgaccatctacagctttccggcgcccaacgtgattctgacgaagccagaggtctcagaagggaccgaggtgacagtgaagtgtgaggcccaccctagagccaaggtgacgctgaatggggttccagcccagccactgggcccgagggcccagctcctgctgaaggccaccccagaggacaacgggcgcagcttctcctgctctgcaaccctggaggtggccggccagcttatacacaagaaccagacccgggagcttcgtgtcctgtatggcccccgactggacgagagggattgtccgggaaactggacgtggccagaaaattcccagcagactccaatgtgccaggcttgggggaacccattgcccgagctcaagtgtctaaaggatggcactttcccactgcccatcggggaatcagtgactgtcactcgagatcttgagggcacctacctctgtcgggccaggagcactcaaggggaggtcacccgcaaggtgaccgtgaatgtgctctccccccggtatgagattgtcatcatcactgtggtagcagccgcagtcataatgggcactgcaggcctcagcacgtacctctataaccgccagcggaagatcaagaaatacagactacaacaggcccaaaaagggacccccatgaaaccgaacacacaagccacgcctccctga

SEQ ID NO: 4 - RNA, 19 nt, synthetic construct
  source 1..19: mol_type = other RNA; note = siRNA of hICAM-1 mRNA
ccaatgtgctattcaaact

SEQ ID NO: 5 - RNA, 19 nt, synthetic construct
  source 1..19: mol_type = other RNA; note = siRNA of hICAM-1 mRNA
agtttgaatagcacattgg

SEQ ID NO: 6 - RNA, 19 nt, synthetic construct
  source 1..19: mol_type = other RNA; note = siRNA of hICAM-1 mRNA
gcctcagtcagtgtgaccg

SEQ ID NO: 7 - RNA, 19 nt, synthetic construct
  source 1..19: mol_type = other RNA; note = siRNA of hICAM-1 mRNA
cggtcacactgactgaggc